European Patent Application EP 4 159 746 A1, published April 5, 2023. Title: A STRUCTURALLY MODIFIED CHIMERIC POLYPEPTIDE OF HPV, A RECOMBINANT PROTEIN COMPRISING THE SAME, AND USE OF THE SAME. Applicant: Genematrix Inc. The sequence listing filed with the application follows.

SEQUENCE LISTING (9 sequences)

SEQ ID NO: 1 - protein, 258 aa, Artificial Sequence
  Chimera polypeptide
MPGDTPTLHEYMLDLQPETTDLYGYEQLNDSSEEEDEMHQKRTAMFQDPQERPRKLPQLCTELQTTIHDIILECVYCKQQLLRREVYDFARRDGCIVYRDGNPYAVCDKCLKFYSKISEYRHYCYSLYGTTLEQQYNKPLCDLLIRCINCQKPLCPEEKQRHLDKKQRFHNIRGRWTGRCMSCCRSSRTRREEEEDEIDGPAGQAEPDRAHYNIVTFCCKCDSTLRLCVQSTHVDIRTLRRLLMGTLGIVCPICSQKP

SEQ ID NO: 2 - DNA, 774 bp, Artificial Sequence
  Polynucleotide encoding Chimera polypeptide
atgccgggcgacacgccgaccttacatgagtacatgcttgatttacagccggaaacgaccgatttatacggttacgaacagttgaacgactctagcgaggaagaagacgagatgcatcaaaaacgcaccgccatgttccaagatccgcaagaacgtccgcgcaaactgccgcagctttgcaccgagctgcaaactaccattcatgacattatccttgagtgcgtgtactgtaaacagcaattattgcgtcgcgaagtatacgacttcgcgcgccgtgacggttgtattgtgtaccgtgacggtaacccgtatgcagtctgcgacaaatgcctgaagttttacagcaagataagcgagtaccgtcattattgttattctttgtatggcaccacccttgagcagcagtacaataagccgctttgtgatttgttgatccgttgcattaattgccagaaaccgttgtgcccggaagaaaagcagcgccatttagacaagaagcagcgtttccataatattcgcgggcgctggaccggtcgttgtatgagctgttgccgttctagccgcactcgtcgtgaagaggaagaagacgagattgacggtccggcagggcaggccgagccggatcgcgctcattataatatcgtgactttttgttgtaagtgtgatagcacccttcgcctttgtgtgcaaagcacccatgttgacattcgtactttgcgccgcttattaatgggcacgcttggtattgtgtgcccgatctgctctcagaagccg

SEQ ID NO: 3 - protein, 256 aa, Artificial Sequence
  Salmonella typhimurium str. LT2, Flagellin (FliC) modified amino acid sequence
MAQVINTNSLSLLTQNNLNKSQSALGTAIERLSSGLRINSAKDDAAGQAIANRFTANIKGLTQASRNANDGISIAQTTEGALNEINNNLQRVRELAVQSANSTNSQSDLDSIQAEITQRLNEIDRVSGQTQFNGVKVLAQDNTGGGGSGGGGSGSGGKLGGGGSGGGGSLQKIDAALAQVDTLRSDLGAVQNRFNSAITNLGNTVNNLTSARSRIEDSDYATEVSNMSRAQILQQAGTSVLAQANQVPQNVLSLLR

SEQ ID NO: 4 - DNA, 768 bp, Artificial Sequence
  polynucleotide encoding Salmonella typhimurium str. LT2, Flagellin (FliC) modified amino acid sequence
atggcgcaggttattaacaccaatagcttatctttgcttacccagaataacttaaacaaatctcaaagcgctcttgggacggcaatcgagcgtttatctagcgggctgcgcattaattctgctaaagacgacgcggcaggtcaagcaatcgccaaccgtttcacggcaaacattaagggccttacccaagccagccgtaatgctaacgacgggatctctatcgcgcagaccaccgaaggcgctctgaacgagatcaacaacaacttgcagcgcgttcgtgagttagcggtgcaatctgccaacagcacgaatagccaatctgacttagacagcatccaggccgagatcacccagcgtcttaatgaaattgatcgcgtatctggccagacgcaatttaacggggtcaaggttcttgcgcaagataataccggtggcggtggttctggtgggggcggcagcggatccggcggtaagcttggtgggggcggcagcggcggtggcggttctttgcagaaaattgacgcggcacttgcgcaggtcgacacccttcgcagtgacctgggggcagttcagaaccgctttaattctgccattacgaacctggggaacactgtgaacaaccttacgtctgcgcgctctcgcatcgaggactctgattatgcaactgaagtgagcaatatgagccgcgcccaaatcttgcagcaggcaggcaccagcgttcttgcccaggcaaaccaagttccgcaaaatgtcctttctcttcttcgt

SEQ ID NO: 5 - protein, 520 aa, Artificial Sequence
  FliC. HPV16 E6, E7 modified amino acid sequence
MAQVINTNSLSLLTQNNLNKSQSALGTAIERLSSGLRINSAKDDAAGQAIANRFTANIKGLTQASRNANDGISIAQTTEGALNEINNNLQRVRELAVQSANSTNSQSDLDSIQAEITQRLNEIDRVSGQTQFNGVKVLAQDNTGGGGSGGGGSGSGGLQMPGDTPTLHEYMLDLQPETTDLYGYEQLNDSSEEEDEMHQKRTAMFQDPQERPRKLPQLCTELQTTIHDIILECVYCKQQLLRREVYDFARRDGCIVYRDGNPYAVCDKCLKFYSKISEYRHYCYSLYGTTLEQQYNKPLCDLLIRCINCQKPLCPEEKQRHLDKKQRFHNIRGRWTGRCMSCCRSSRTRREEEEDEIDGPAGQAEPDRAHYNIVTFCCKCDSTLRLCVQSTHVDIRTLRRLLMGTLGIVCPICSQKPQLGGKLGGGGSGGGGSLQKIDAALAQVDTLRSDLGAVQNRFNSAITNLGNTVNNLTSARSRIEDSDYATEVSNMSRAQILQQAGTSVLAQANQVPQNVLSLLR

SEQ ID NO: 6 - DNA, 1560 bp, Artificial Sequence
  FliC. HPV16 E6, E7 modified nucleic acid sequence
atggcgcaggttattaacaccaatagcttatctttgcttacccagaataacttaaacaaatctcaaagcgctcttgggacggcaatcgagcgtttatctagcgggctgcgcattaattctgctaaagacgacgcggcaggtcaagcaatcgccaaccgtttcacggcaaacattaagggccttacccaagccagccgtaatgctaacgacgggatctctatcgcgcagaccaccgaaggcgctctgaacgagatcaacaacaacttgcagcgcgttcgtgagttagcggtgcaatctgccaacagcacgaatagccaatctgacttagacagcatccaggccgagatcacccagcgtcttaatgaaattgatcgcgtatctggccagacgcaatttaacggggtcaaggttcttgcgcaagataataccggtggcggtggttctggtgggggcggcagcggatccggcggtctgcagatgccgggcgacacgccgaccttacatgagtacatgcttgatttacagccggaaacgaccgatttatacggttacgaacagttgaacgactctagcgaggaagaagacgagatgcatcaaaaacgcaccgccatgttccaagatccgcaagaacgtccgcgcaaactgccgcagctttgcaccgagctgcaaactaccattcatgacattatccttgagtgcgtgtactgtaaacagcaattattgcgtcgcgaagtatacgacttcgcgcgccgtgacggttgtattgtgtaccgtgacggtaacccgtatgcagtctgcgacaaatgcctgaagttttacagcaagataagcgagtaccgtcattattgttattctttgtatggcaccacccttgagcagcagtacaataagccgctttgtgatttgttgatccgttgcattaattgccagaaaccgttgtgcccggaagaaaagcagcgccatttagacaagaagcagcgtttccataatattcgcgggcgctggaccggtcgttgtatgagctgttgccgttctagccgcactcgtcgtgaagaggaagaagacgagattgacggtccggcagggcaggccgagccggatcgcgctcattataatatcgtgactttttgttgtaagtgtgatagcacccttcgcctttgtgtgcaaagcacccatgttgacattcgtactttgcgccgcttattaatgggcacgcttggtattgtgtgcccgatctgctctcagaagccgcaattgggtggcaagcttggtgggggcggcagcggcggtggcggttctttgcagaaaattgacgcggcacttgcgcaggtcgacacccttcgcagtgacctgggggcagttcagaaccgctttaattctgccattacgaacctggggaacactgtgaacaaccttacgtctgcgcgctctcgcatcgaggactctgattatgcaactgaagtgagcaatatgagccgcgcccaaatcttgcagcaggcaggcaccagcgttcttgcccaggcaaaccaagttccgcaaaatgtcctttctcttcttcgt

SEQ ID NO: 7 - DNA, 30 bp, Artificial Sequence
  Forward primer
cgacgcgcatatgatgcatcaaaaacgcac

SEQ ID NO: 8 - DNA, 27 bp, Artificial Sequence
  Forward primer
gaacgcgcatatgatgccgggcgacac

SEQ ID NO: 9 - DNA, 30 bp, Artificial Sequence
  Reverse primer
ctcgcctcgagttacggcttctgagagcag